European Patent Application EP 4 269 571 A1, published November 1, 2023. Title: Method for producing naive human iPS cells from somatic cells. Applicant: KYOTO UNIVERSITY ID PHARMA CO., LTD. The sequence listing filed with the application follows.

SEQUENCE LISTING (1 sequence)

SEQ ID NO: 1 - DNA, 48 bp, Artificial Sequence
  Synthetic polynucleotide
tcaccattgctaaagtgcaattcgattcaccattgctaaagtgcaatt